European Patent Application EP 4 752 885 A1, published June 3, 2026. Title: A Computer-Implemented Method for Preparing Alignment Information an Oligonucleotide Sequence to a Target Nucleic Acid Sequence. Applicant: Seegene, Inc. The sequence listing filed with the application follows.

SEQUENCE LISTING (17 sequences)

SEQ ID NO: 1 - DNA, 13 bp, unidentified
  source 1..13: mol_type = genomic DNA
tcagccagctgca

SEQ ID NO: 2 - skipped

SEQ ID NO: 3 - DNA, 23 bp, synthetic construct
  source 1..23: mol_type = other DNA
ctgcagatttggatgatttctcc

SEQ ID NO: 4 - DNA, 23 bp, SARS-CoV-2
  source 1..23: mol_type = genomic DNA
ctgcagatttggatgatttctcc

SEQ ID NO: 5 - DNA, 23 bp, SARS-CoV-2
  source 1..23: mol_type = genomic DNA
tttaggatttggatgatctatgt

SEQ ID NO: 6 - DNA, 23 bp, SARS-CoV-2
  source 1..23: mol_type = genomic DNA
ctgtagatttggatgatttctcc

SEQ ID NO: 7 - DNA, 23 bp, SARS-CoV-2
  source 1..23: mol_type = genomic DNA
ctgcagatttgtatgatttctcc

SEQ ID NO: 8 - DNA, 23 bp, SARS-CoV-2
  source 1..23: mol_type = genomic DNA
gtacagaagtaaatgagttcgcc

SEQ ID NO: 9 - DNA, 24 bp, SARS-CoV-2
  source 1..24: mol_type = genomic DNA
ctttaggatttggatgatctatgt

SEQ ID NO: 10 - DNA, 40 bp, synthetic construct
  source 1..40: mol_type = other DNA
  modified_base 26..30: mod_base = i
gactctagagagactgccgtcgtaannnnngaggaaggtg

SEQ ID NO: 11 - DNA, 40 bp, Bacteroides fragilis
  source 1..40: mol_type = genomic DNA
gactctggagagactgccgtcgtaagatgtgaggaaggtg

SEQ ID NO: 12 - DNA, 40 bp, Bacteroides fragilis
  source 1..40: mol_type = genomic DNA
gattctatagtgattgccgtaaagtcgggattgaaagata

SEQ ID NO: 13 - DNA, 40 bp, Bacteroides fragilis
  source 1..40: mol_type = genomic DNA
cctcaaggagagactgcatatttcgaagaaagcgcacctc

SEQ ID NO: 14 - DNA, 40 bp, Bacteroides fragilis
  source 1..40: mol_type = genomic DNA
atctttacagagactgccgatcaggaaaaagagcatgcaa

SEQ ID NO: 15 - DNA, 40 bp, Bacteroides fragilis
  source 1..40: mol_type = genomic DNA
gactctagagagactgccgtcgtaagatgtgaggaaggtg

SEQ ID NO: 16 - DNA, 40 bp, Bacteroides fragilis
  source 1..40: mol_type = genomic DNA
gagtaaagacagactgtcggcaaaatctttgtagaagtcg

SEQ ID NO: 17 - DNA, 39 bp, Bacteroides fragilis
  source 1..39: mol_type = genomic DNA
aacttcggggagactatcctttaagaagagaggaaggtg